European Patent Application EP 4 772 615 A1, published July 8, 2026. Title: A recombinant oncolytic adeno virus. Applicant: Osaka University. Application IB. The sequence listing filed with the application follows.

SEQUENCE LISTING (4 sequences)

SEQ ID NO: 1 - DNA, 1429 bp, Human adenovirus 5
  source 1..1429: mol_type = genomic DNA
tcacagaaccctagtattcaacctgccacctccctcccaacacacagagtacacagtcctttctccccggctggccttaaaaagcatcatatcatgggtaacagacatattcttaggtgttatattccacacggtttcctgtcgagccaaacgctcatcagtgatattaataaactccccgggcagctcacttaagttcatgtcgctgtccagctgctgagccacaggctgctgtccaacttgcggttgcttaacgggcggcgaaggagaagtccacgcctacatgggggtagagtcataatcgtgcatcaggatagggcggtggtgctgcagcagcgcgcgaataaactgctgccgccgccgctccgtcctgcaggaatacaacatggcagtggtctcctcagcgatgattcgcaccgcccgcagcataaggcgccttgtcctccgggcacagcagcgcaccctgatctcacttaaatcagcacagtaactgcagcacagcaccacaatattgttcaaaatcccacagtgcaaggcgctgtatccaaagctcatggcggggaccacagaacccacgtggccatcataccacaagcgcaggtagattaagtggcgacccctcataaacacgctggacataaacattacctcttttggcatgttgtaattcaccacctcccggtaccatataaacctctgattaaacatggcgccatccaccaccatcctaaaccagctggccaaaacctgcccgccggctatacactgcagggaaccgggactggaacaatgacagtggagagcccaggactcgtaaccatggatcatcatgctcgtcatgatatcaatgttggcacaacacaggcacacgtgcatacacttcctcaggattacaagctcctcccgcgttagaaccatatcccagggaacaacccattcctgaatcagcgtaaatcccacactgcagggaagacctcgcacgtaactcacgttgtgcattgtcaaagtgttacattcgggcagcagcggatgatcctccagtatggtagcgcgggtttctgtctcaaaaggaggtagacgatccctactgtacggagtgcgccgagacaaccgagatcgtgttggtcgtagtgtcatgccaaatggaacgccggacgtagtcatatttcctgaagcaaaaccaggtgcgggcgtgacaaacagatctgcgtctccggtctcgccgcttagatcgctctgtgtagtagttgtagtatatccactctctcaaagcatccaggcgccccctggcttcgggttctatgtaaactccttcatgcgccgctgccctgataacatccaccaccgcagaataagccacacccagccaacctacacattcgttctgcgagtcacacacgggaggagcgggaagagctggaagaaccat

SEQ ID NO: 2 - DNA, 2950 bp, Human adenovirus 5
  source 1..2950: mol_type = genomic DNA
atgagacatattatctgccacggaggtgttattaccgaagaaatggccgccagtcttttggaccagctgatcgaagaggtactggctgataatcttccacctcctagccattttgaaccacctacccttcacgaactgtatgatttagacgtgacggcccccgaagatcccaacgaggaggcggtttcgcagatttttcccgactctgtaatgttggcggtgcaggaagggattgacttactcacttttccgccggcgcccggttctccggagccgcctcacctttcccggcagcccgagcagccggagcagagagccttgggtccggtttctatgccaaaccttgtaccggaggtgatcgatcttacctgccacgaggctggctttccacccagtgacgacgaggatgaagagggtgaggagtttgtgttagattatgtggagcaccccgggcacggttgcaggtcttgtcattatcaccggaggaatacgggggacccagatattatgtgttcgctttgctatatgaggacctgtggcatgtttgtctacagtaagtgaaaattatgggcagtgggtgatagagtggtgggtttggtgtggtaattttttttttaatttttacagttttgtggtttaaagaattttgtattgtgatttttttaaaaggtcctgtgtctgaacctgagcctgagcccgagccagaaccggagcctgcaagacctacccgccgtcctaaaatggcgcctgctatcctgagacgcccgacatcacctgtgtctagagaatgcaatagtagtacggatagctgtgactccggtccttctaacacacctcctgagatacacccggtggtcccgctgtgccccattaaaccagttgccgtgagagttggtgggcgtcgccaggctgtggaatgtatcgaggacttgcttaacgagcctgggcaacctttggacttgagctgtaaacgccccaggccataaggtgtaaacctgtgattgcgtgtgtggttaacgcctttgtttgctgaatgagttgatgtaagtttaataaagggtgagataatgtttaacttgcatggcgtgttaaatggggcggggcttaaagggtatataatgcgccgtgggctaatcttggttacatctgacctcatggaggcttgggagtgtttggaagatttttctgctgtgcgtaacttgctggaacagagctctaacagtacctcttggttttggaggtttctgtggggctcatcccaggcaaagttagtctgcagaattaaggaggattacaagtgggaatttgaagagcttttgaaatcctgtggtgagctgtttgattctttgaatctgggtcaccaggcgcttttccaagagaaggtcatcaagactttggatttttccacaccggggcgcgctgcggctgctgttgcttttttgagttttataaaggataaatggagcgaagaaacccatctgagcggggggtacctgctggattttctggccatgcatctgtggagagcggttgtgagacacaagaatcgcctgctactgttgtcttccgtccgcccggcgataataccgacggaggagcagcagcagcagcaggaggaagccaggcggcggcggcaggagcagagcccatggaacccgagagccggcctggaccctcgggaatgaatgttgtacaggtggctgaactgtatccagaactgagacgcattttgacaattacagaggatgggcaggggctaaagggggtaaagagggagcggggggcttgtgaggctacagaggaggctaggaatctagcttttagcttaatgaccagacaccgtcctgagtgtattacttttcaacagatcaaggataattgcgctaatgagcttgatctgctggcgcagaagtattccatagagcagctgaccacttactggctgcagccaggggatgattttgaggaggctattagggtatatgcaaaggtggcacttaggccagattgcaagtacaagatcagcaaacttgtaaatatcaggaattgttgctacatttctgggaacggggccgaggtggagatagatacggaggatagggtggcctttagatgtagcatgataaatatgtggccgggggtgcttggcatggacggggtggttattatgaatgtaaggtttactggccccaattttagcggtacggttttcctggccaataccaaccttatcctacacggtgtaagcttctatgggtttaacaatacctgtgtggaagcctggaccgatgtaagggttcggggctgtgccttttactgctgctggaagggggtggtgtgtcgccccaaaagcagggcttcaattaagaaatgcctctttgaaaggtgtaccttgggtatcctgtctgagggtaactccagggtgcgccacaatgtggcctccgactgtggttgcttcatgctagtgaaaagcgtggctgtgattaagcataacatggtatgtggcaactgcgaggacagggcctctcagatgctgacctgctcggacggcaactgtcacctgctgaagaccattcacgtagccagccactctcgcaaggcctggccagtgtttgagcataacatactgacccgctgttccttgcatttgggtaacaggaggggggtgttcctaccttaccaatgcaatttgagtcacactaagatattgcttgagcccgagagcatgtccaaggtgaacctgaacggggtgtttgacatgaccatgaagatctggaaggtgctgaggtacgatgagacccgcaccaggtgcagaccctgcgagtgtggcggtaaacatattaggaaccagcctgtgatgctggatgtgaccgaggagctgaggcccgatcacttggtgctggcctgcacccgcgctgagtttggctctagcgatgaagatacagattga

SEQ ID NO: 3 - DNA, 15 bp, Human adenovirus 5
  source 1..15: mol_type = genomic DNA
cttacctgccacgag

SEQ ID NO: 4 - DNA, 15 bp, Human adenovirus 5
  source 1..15: mol_type = other DNA
gttacctcccacgat